European Patent Application EP 4 755 394 A1, published June 10, 2026. Title: 一种新型多肽、多肽衍生物及其应用. Applicant: 南京安吉生物科技有限公司. Application CN. The sequence listing filed with the application follows.

SEQUENCE LISTING (53 sequences)

SEQ ID NO: 1 - protein, 51 aa, synthetic construct
MERAGVPGFSPRRSSVEAKMQSTSCSVRKSSTVTAWPAVVLLLSWGQRRGG

SEQ ID NO: 2 - protein, 48 aa, synthetic construct
AGVPGFSPRRSSVEAKMQSTSCSVRKSSTVTAWPAVVLLLSWGQRRGG

SEQ ID NO: 3 - protein, 48 aa, synthetic construct
MERPGFSPRRSSVEAKMQSTSCSVRKSSTVTAWPAVVLLLSWGQRRGG

SEQ ID NO: 4 - protein, 48 aa, synthetic construct
MERAGVSPRRSSVEAKMQSTSCSVRKSSTVTAWPAVVLLLSWGQRRGG

SEQ ID NO: 5 - protein, 48 aa, synthetic construct
MERAGVPGFRSSVEAKMQSTSCSVRKSSTVTAWPAVVLLLSWGQRRGG

SEQ ID NO: 6 - protein, 48 aa, synthetic construct
MERAGVPGFSPRVEAKMQSTSCSVRKSSTVTAWPAVVLLLSWGQRRGG

SEQ ID NO: 7 - protein, 48 aa, synthetic construct
MERAGVPGFSPRRSSKMQSTSCSVRKSSTVTAWPAVVLLLSWGQRRGG

SEQ ID NO: 8 - protein, 48 aa, synthetic construct
MERAGVPGFSPRRSSVEASTSCSVRKSSTVTAWPAVVLLLSWGQRRGG

SEQ ID NO: 9 - protein, 48 aa, synthetic construct
MERAGVPGFSPRRSSVEAKMQCSVRKSSTVTAWPAVVLLLSWGQRRGG

SEQ ID NO: 10 - protein, 48 aa, synthetic construct
MERAGVPGFSPRRSSVEAKMQSTSRKSSTVTAWPAVVLLLSWGQRRGG

SEQ ID NO: 11 - protein, 48 aa, synthetic construct
MERAGVPGFSPRRSSVEAKMQSTSCSVSTVTAWPAVVLLLSWGQRRGG

SEQ ID NO: 12 - protein, 48 aa, synthetic construct
MERAGVPGFSPRRSSVEAKMQSTSCSVRKSTAWPAVVLLLSWGQRRGG

SEQ ID NO: 13 - protein, 48 aa, synthetic construct
MERAGVPGFSPRRSSVEAKMQSTSCSVRKSSTVPAVVLLLSWGQRRGG

SEQ ID NO: 14 - protein, 48 aa, synthetic construct
MERAGVPGFSPRRSSVEAKMQSTSCSVRKSSTVTAWVLLLSWGQRRGG

SEQ ID NO: 15 - protein, 48 aa, synthetic construct
MERAGVPGFSPRRSSVEAKMQSTSCSVRKSSTVTAWPAVLSWGQRRGG

SEQ ID NO: 16 - protein, 48 aa, synthetic construct
MERAGVPGFSPRRSSVEAKMQSTSCSVRKSSTVTAWPAVVLLGQRRGG

SEQ ID NO: 17 - protein, 48 aa, synthetic construct
MERAGVPGFSPRRSSVEAKMQSTSCSVRKSSTVTAWPAVVLLLSWRGG

SEQ ID NO: 18 - protein, 48 aa, synthetic construct
MERAGVPGFSPRRSSVEAKMQSTSCSVRKSSTVTAWPAVVLLLSWGQR

SEQ ID NO: 19 - protein, 47 aa, synthetic construct
GVPGFSPRRSSVEAKMQSTSCSVRKSSTVTAWPAVVLLLSWGQRRGG

SEQ ID NO: 20 - protein, 42 aa, synthetic construct
SPRRSSVEAKMQSTSCSVRKSSTVTAWPAVVLLLSWGQRRGG

SEQ ID NO: 21 - protein, 37 aa, synthetic construct
SVEAKMQSTSCSVRKSSTVTAWPAVVLLLSWGQRRGG

SEQ ID NO: 22 - protein, 32 aa, synthetic construct
MQSTSCSVRKSSTVTAWPAVVLLLSWGQRRGG

SEQ ID NO: 23 - protein, 27 aa, synthetic construct
CSVRKSSTVTAWPAVVLLLSWGQRRGG

SEQ ID NO: 24 - protein, 22 aa, synthetic construct
SSTVTAWPAVVLLLSWGQRRGG

SEQ ID NO: 25 - protein, 17 aa, synthetic construct
AWPAVVLLLSWGQRRGG

SEQ ID NO: 26 - protein, 51 aa, synthetic construct
MARAGVPGFSPRRSSVEAKMQSTSCSVRKSSTVTAWPAVVLLLSWGQRRGG

SEQ ID NO: 27 - protein, 51 aa, synthetic construct
MEAAGVPGFSPRRSSVEAKMQSTSCSVRKSSTVTAWPAVVLLLSWGQRRGG

SEQ ID NO: 28 - protein, 51 aa, synthetic construct
MERAGVPAFSPRRSSVEAKMQSTSCSVRKSSTVTAWPAVVLLLSWGQRRGG

SEQ ID NO: 29 - protein, 51 aa, synthetic construct
MERAGVPGASPRRSSVEAKMQSTSCSVRKSSTVTAWPAVVLLLSWGQRRGG

SEQ ID NO: 30 - protein, 51 aa, synthetic construct
MERAGVPGFAPRRSSVEAKMQSTSCSVRKSSTVTAWPAVVLLLSWGQRRGG

SEQ ID NO: 31 - protein, 51 aa, synthetic construct
MERAGVPGFSARRSSVEAKMQSTSCSVRKSSTVTAWPAVVLLLSWGQRRGG

SEQ ID NO: 32 - protein, 51 aa, synthetic construct
MERAGVPGFSPARSSVEAKMQSTSCSVRKSSTVTAWPAVVLLLSWGQRRGG

SEQ ID NO: 33 - protein, 51 aa, synthetic construct
MERAGVPGFSPRASSVEAKMQSTSCSVRKSSTVTAWPAVVLLLSWGQRRGG

SEQ ID NO: 34 - protein, 51 aa, synthetic construct
MERAGVPGFSPRRSSVAAKMQSTSCSVRKSSTVTAWPAVVLLLSWGQRRGG

SEQ ID NO: 35 - protein, 51 aa, synthetic construct
MERAGVPGFSPRRSSVEAAMQSTSCSVRKSSTVTAWPAVVLLLSWGQRRGG

SEQ ID NO: 36 - protein, 51 aa, synthetic construct
MERAGVPGFSPRRSSVEAKAQSTSCSVRKSSTVTAWPAVVLLLSWGQRRGG

SEQ ID NO: 37 - protein, 51 aa, synthetic construct
MERAGVPGFSPRRSSVEAKMASTSCSVRKSSTVTAWPAVVLLLSWGQRRGG

SEQ ID NO: 38 - protein, 51 aa, synthetic construct
MERAGVPGFSPRRSSVEAKMQATSCSVRKSSTVTAWPAVVLLLSWGQRRGG

SEQ ID NO: 39 - protein, 51 aa, synthetic construct
MERAGVPGFSPRRSSVEAKMQSTSASVRKSSTVTAWPAVVLLLSWGQRRGG

SEQ ID NO: 40 - protein, 51 aa, synthetic construct
MERAGVPGFSPRRSSVEAKMQSTSCSARKSSTVTAWPAVVLLLSWGQRRGG

SEQ ID NO: 41 - protein, 51 aa, synthetic construct
MERAGVPGFSPRRSSVEAKMQSTSCSVAKSSTVTAWPAVVLLLSWGQRRGG

SEQ ID NO: 42 - protein, 51 aa, synthetic construct
MERAGVPGFSPRRSSVEAKMQSTSCSVRKASTVTAWPAVVLLLSWGQRRGG

SEQ ID NO: 43 - protein, 51 aa, synthetic construct
MERAGVPGFSPRRSSVEAKMQSTSCSVRKSATVTAWPAVVLLLSWGQRRGG

SEQ ID NO: 44 - protein, 51 aa, synthetic construct
MERAGVPGFSPRRSSVEAKMQSTSCSVRKSSAVTAWPAVVLLLSWGQRRGG

SEQ ID NO: 45 - protein, 51 aa, synthetic construct
MERAGVPGFSPRRSSVEAKMQSTSCSVRKSSTVTAWPAVALLLSWGQRRGG

SEQ ID NO: 46 - protein, 51 aa, synthetic construct
MERAGVPGFSPRRSSVEAKMQSTSCSVRKSSTVTAWPAVVALLSWGQRRGG

SEQ ID NO: 47 - protein, 51 aa, synthetic construct
MERAGVPGFSPRRSSVEAKMQSTSCSVRKSSTVTAWPAVVLALSWGQRRGG

SEQ ID NO: 48 - protein, 51 aa, synthetic construct
MERAGVPGFSPRRSSVEAKMQSTSCSVRKSSTVTAWPAVVLLASWGQRRGG

SEQ ID NO: 49 - protein, 51 aa, synthetic construct
MERAGVPGFSPRRSSVEAKMQSTSCSVRKSSTVTAWPAVVLLLAWGQRRGG

SEQ ID NO: 50 - protein, 51 aa, synthetic construct
MERAGVPGFSPRRSSVEAKMQSTSCSVRKSSTVTAWPAVVLLLSAGQRRGG

SEQ ID NO: 51 - protein, 51 aa, synthetic construct
MERAGVPGFSPRRSSVEAKMQSTSCSVRKSSTVTAWPAVVLLLSWGQARGG

SEQ ID NO: 52 - protein, 51 aa, synthetic construct
MERAGVPGFSPRRSSVEAKMQSTSCSVRKSSTVTAWPAVVLLLSWGQRAGG

SEQ ID NO: 53 - protein, 51 aa, synthetic construct
MERAGVPGFSPRRSSVEAKMQSTSCSVRKSSTVTAWPAVVLLLSWGQRRAG